European Patent Application EP 4 166 679 A1, published April 19, 2023. Title: A line elimination lateral flow immunochromatographic strip and its application in crispr nucleic acid detection. Applicant: Academy of Military Medical Sciences. Application 21823030.8. The sequence listing filed with the application follows.

SEQUENCE LISTING (12 sequences)

SEQ ID NO: 1 - RNA, 20 nt, Artificial sequence
uuuuuuuuuuuuuuuuuuuu

SEQ ID NO: 2 - RNA, 66 nt, Artificial sequence
gggauuuagacuaccccaaaaacgaaggggacuaaaacuccaauuugauggcaccuguguagguca

SEQ ID NO: 3 - DNA, 55 bp, Artificial sequence
aattctaatacgactcactatagggaactaatcagacaaggaactgattacaaac

SEQ ID NO: 4 - DNA, 30 bp, Artificial sequence
cttattcagcaaaatgacttgatctttgaa

SEQ ID NO: 5 - RNA, 66 nt, Artificial sequence
gggauuuagacuaccccaaaaacgaaggggacuaaaacauuguaucaguccuugcucugcauguac

SEQ ID NO: 6 - DNA, 55 bp, Artificial sequence
aattctaatacgactcactatagggtagtaggagaaaaggcttgccttgagaagg

SEQ ID NO: 7 - DNA, 31 bp, Artificial sequence
tgttcgcatcaaacggaaaatcaccatcatg

SEQ ID NO: 8 - RNA, 66 nt, Artificial sequence
gggauuuagacuaccccaaaaacgaaggggacuaaaacgaugguggcucagggagaacaagaaccg

SEQ ID NO: 9 - DNA, 57 bp, Artificial sequence
aattctaatacgactcactatagggagggaagagagaaattggcaactctcttcagg

SEQ ID NO: 10 - DNA, 31 bp, Artificial sequence
tccgagtcacacgtcacctccttgtcagact

SEQ ID NO: 11 - DNA, 54 bp, Artificial sequence
aattctaatacgactcactatagggaattgcacaatttgcccccagcgcttcag

SEQ ID NO: 12 - DNA, 30 bp, Artificial sequence
cttgatctttgaaatttggatctttgtcat